European Patent Application EP 4 772 642 A1, published July 8, 2026. Title: 用于非B型DNA序列的克隆/表达载体. Applicant: 南京金斯瑞生物科技有限公司. Application CN. The sequence listing filed with the application follows.

SEQUENCE LISTING (29 sequences)

SEQ ID NO: 1 - DNA, 99 bp, synthetic construct
  source 1..99: mol_type = other DNA
ggaagagcctagctacctactcgagtctagagggcccgtttaaacctcagatcattgtcacatgtgagcggccaggaaccgtggccgcgttgctggcgt

SEQ ID NO: 2 - DNA, 247 bp, synthetic construct
  source 1..247: mol_type = other DNA
ggaagagcctagctacctactcgagtctagagggcccgtttaaacccgctgatcagcctcgactctagcttggatggaagacgccaaaaacataaagaaaggcccggcgccattctatccgctggaagatggaaccgctggagagcaactgcataaggctatgaagagcaagctcagatcattgtcacatgtgagcaaaaggccagcaaaaggccaggaaccgtaaaaaggccgcgttgctggcgtt

SEQ ID NO: 3 - DNA, 500 bp, synthetic construct
  source 1..500: mol_type = other DNA
ggaagagcctagctacctactcgagtctagaatggaagacgccaaaaacataaagaaaggcccggcgccattctatccgctggaagatggaaccgctggagagcaactgcataaggctatgaagagatacgccctggttcctggaacaattgcttttacagatgcacatatcgaggtggacatcacttacgctgagtacttcgaaatgtccgttcggttggcagaagctatgaaacgatatgggctgaatacaaatcacagaatcgtcgtatgcagtgaaaactctcttcaattctttatgccggtgttgggcgcgttatttatcggagttgcagttgcgcccgcgaacgacatttataatgaacgtgaattgctcaacagtatgggcatttcgcagcctaccgtggtgttcgtttccaaaaaggggttgcaaaaaattacatgtgagcaaaaggccagcaaaaggccaggaaccgtaaaaaggccgcgttgctggcgtt

SEQ ID NO: 4 - DNA, 700 bp, synthetic construct
  source 1..700: mol_type = other DNA
ggaagagcctagctacctactcgagtctagaatggaagacgccaaaaacataaagaaaggcccggcgccattctatccgctggaagatggaaccgctggagagcaactgcataaggctatgaagagatacgccctggttcctggaacaattgcttttacagatgcacatatcgaggtggacatcacttacgctgagtacttcgaaatgtccgttcggttggcagaagctatgaaacgatatgggctgaatacaaatcacagaatcgtcgtatgcagtgaaaactctcttcaattctttatgccggtgttgggcgcgttatttatcggagttgcagttgcgcccgcgaacgacatttataatgaacgtgaattgctcaacagtatgggcatttcgcagcctaccgtggtgttcgtttccaaaaaggggttgcaaaaaattttgaacgtgcaaaaaaagctcccaatcatccaaaaaattattatcatggattctaaaacggattaccagggatttcagtcgatgtacacgttcgtcacatctcatctacctcccggttttaatgaatacgattttgtgccagagtccttcgatagggacaagacaattgcactgatcatgaactcctctggatctactggacatgtgagcaaaaggccagcaaaaggccaggaaccgtaaaaaggccgcgttgctggcgtt

SEQ ID NO: 5 - DNA, 247 bp, synthetic construct
  source 1..247: mol_type = other DNA
ggaagagcctagctacctactcgagtctagagggcccgtttaaacccgctgatcagcctcgactctagcttggattctcaccaataaaaaacgcccggcggcaaccgagcgttctgaacaaatccagatggagttctgaggtcattactggatctatcaacaggagtccaagctcagatcattgtcacatgtgagcaaaaggccagcaaaaggccaggaaccgtaaaaaggccgcgttgctggcgtt

SEQ ID NO: 6 - DNA, 465 bp, synthetic construct
  source 1..465: mol_type = other DNA
ggaagagcctagctacctactcgagtctagaatggaagacgccaaaaacataaagaaaggcccggcgccattctatccgctggaagatggaaccgctggagagcaactgcataaggctatgaagagatacgccctggttcctggaacaattgcttttacagatgcacatatcgaggtggacatcacttacgctgagtacttcgaaatgtccgttcggttggcagaagctatgaaacgatatgggctgaatacaaatcacagaatcgtcgtatgcagtgaaaactctcttcaattctttatgccggtgttgggcgcgttattataatgaacgtgaattgctcaacagtatgggcatttcgcagcctaccgtggtgttcgtttccaaaaaggggttgcaaaaaattacatgtgagcaaaaggccagcaaaaggccaggaaccgtaaaaaggccgcgttgctggcgtt

SEQ ID NO: 7 - DNA, 110 bp, synthetic construct
  source 1..110: mol_type = other DNA
gcgcaacgcaattaatgtgagttagctcactcattaggcaccccaggctttacactttatgcttccggctcgtatgttgtgtggaattgtgagcggataacaatttcaca

SEQ ID NO: 8 - DNA, 91 bp, synthetic construct
  source 1..91: mol_type = other DNA
ttgttatccgctcacaattccacacaacatacgagccggaagcataaagtgtaaagcctggggtgcctaatgagtgagctaactcacatta

SEQ ID NO: 9 - DNA, 145 bp, synthetic construct
  source 1..145: mol_type = other DNA
ttggccactccctctctgcgcgctcgctcgctcactgaggccgggcgaccaaaggtcgcccgacgcccgggctttgcccgggcggcctcagtgagcgagcgagcgcgcagagagggagtggccaactccatcactaggggttcct

SEQ ID NO: 10 - DNA, 141 bp, synthetic construct
  source 1..141: mol_type = other DNA
aggaacccctagtgatggagttggccactccctctctgcgcgctcgctcgctcactgaggccgggcgaccaaaggtcgcccgacgcccgggctttgcccgggcggcctcagtgagcgagcgagcgcgcagctgcctgcagg

SEQ ID NO: 11 - DNA, 130 bp, synthetic construct
  source 1..130: mol_type = other DNA
cctgcaggcagctgcgcgctcgctcgctcactgaggccgcccgggcgtcgggcgacctttggtcgcccggcctcagtgagcgagcgagcgcgcagagagggagtggccaactccatcactaggggttcct

SEQ ID NO: 12 - DNA, 128 bp, synthetic construct
  source 1..128: mol_type = other DNA
gcgcgctcgctcgctcactgaggccgggcgaccaaaggtcgcccgacgcccgggctttgcccgggcggcctcagtgagcgagcgagcgcgcagagagggagtggccaactccatcactaggggttcct

SEQ ID NO: 13 - DNA, 110 bp, synthetic construct
  source 1..110: mol_type = other DNA
tctggcgtaccgttcctgtctaaaatccctttaatcggcctcctgtttagctcccgctctgattctaacgaggaaagcacgttatacgtgctcgtcaaagcaacgatagt

SEQ ID NO: 14 - DNA, 4604 bp, synthetic construct
  source 1..4604: mol_type = other DNA
gtcgactagagctcgctgatcagcctcgactgtgccttctagttgccagccatctgttgtttgcccctcccccgtgccttccttgaccctggaaggtgccactcccactgtcctttcctaataaaatgaggaaattgcatcgcattgtctgagtaggtgtcattctattctggggggtggggtggggcaggacagcaagggggaggattggcaagacaatagcaggaaccccactcccacgcgtaggaacccctagtgatggagttggccactccctctctgcgcgctcgctcgctcactgaggccgcccgggcaaagcccgggcgtcgggcgacctttggtcgcccggcctcagtgagcgagcgagcgcgcagagagggagtggccaaggtacctctggccgtcgttttacaacgtcgtgactgggaaaaccctggcgttacccaacttaatcgccttgcagcacatcccgtcagaccccgtagaaaagatcaaaggatcttcttgagatcctttttttctgcgcgtaatctgctgcttgcaaacaaaaaaaccaccgctaccagcggtggtttgtttgccggatcaagagctaccaactctttttccgaaggtaactggcttcagcagagcgcagataccaaatactgttcttctagtgtagccgtagttaggccaccacttcaagaactctgtagcaccgcctacatacctcgctctgctaatcctgttaccagtggctgctgccagtggcgataagtcgtgtcttaccgggttggactcaagacgatagttaccggataaggcgcagcggtcgggctgaacggggggttcgtgcacacagcccagcttggagcgaacgacctacaccgaactgagatacctacagcgtgagctatgagaaagcgccacgcttcccgaagggagaaaggcggacaggtatccggtaagcggcagggtcggaacaggagagcgcacgagggagcttccagggggaaacgcctggtatctttatagtcctgtcgggtttcgccacctctgacttgagcgtcgatttttgtgatgctcgtcaggggggcggagcctatggaaaaacgccagcaacgcggcctttttacggttcctggccttttgctggccttttgctcacatgttctttcctttcgccagctggcgtaatagcgaagaggcccgcaccgatcgcccttcccaacagttgcgcagcatgaatggcgaatggcgcctgatgcggtattttctccttacgcatctgtgcggtatttcacaccgcatatggtgcactctcagtacaatctgctctgatgccgcatagttaagccagccccgacacccgccaacacccgctgacgcgccctgacgggcttgtctgctcccggcatccgcttacagacaagctgtgaccgacgccgggagctgcatgtgtcagaggttttcaccgtcatcaccgaaacgcgcgatgcagctctggcccgtgtctcaaaatctctgatgttacattgcacaagataaaaatatatcatcatgaacaataaaactgtctgcttacataaacagtaatacaaggggtgttatgagccatattcaacgggaaacgtcgaggccgcgattaaattccaacatggatgctgatttatatgggtataaatgggctcgcgataatgtcgggcaatcaggtgcgacaatctatcgcttgtatgggaagcccgatgcgccagagttgtttctgaaacatggcaaaggtagcgttgccaatgatgttacagatgagatggtcagactaaactggctgacggaatttatgcctcttccgaccatcaagcattttatccgtactcctgatgatgcatggttactcaccactgcgatccccggaaaaacagcattccaggtattagaagaatatcctgattcaggtgaaaatattgttgatgcgctggcagtgttcctgcgccggttgcattcgattcctgtttgtaattgtccttttaacagcgatcgcgtatttcgcctcgctcaggcgcaatcacgaatgaataacggtttggttgatgcgagtgattttgatgacgagcgtaatggctggcctgttgaacaagtctggaaagaaatgcataaacttttgccattctcaccggattcagtcgtcactcatggtgatttctcacttgataaccttatttttgacgaggggaaattaataggttgtattgatgttggacgagtcggaatcgcagaccgataccaggatcttgccatcctatggaactgcctcggtgagttttctccttcattacagaaacggctttttcaaaaatatggtattgataatcctgatatgaataaattgcagtttcatttgatgctcgatgagtttttctaactgtcagaccaagtttactcatatatactttagattgatttaaaacttcatttttaatttaaaaggatctaggtgaagatcctttttgataatctcatgaccaaaatcccttaacgtgagttttcgttccactgagcgtcagaccctgcgttatcccctgattctgtggataaccgtattaccgcctttgagtgagctgataccgctcgccgcagccgaacgaccgagcgcagcgagtcagtgagcgaggaagcggaagaacgcccaatacgcaaaccgcctctccccgcgcgttggccgattcattaatgcagctggcacgacaggtttcccgactggaaagcgggcagtgatctggcgtaccgttcctgtctaaaatccctttaatcggcctcctgtttagctcccgctctgattctaacgaggaaagcacgttatacgtgctcgtcaaagcaacgatagtcaggaaacagctatgaccatgattacacccaattgttggccactccctctctgcgcgctcgctcgctcactgaggccgggcgaccaaaggtcgcccgacgcccgggctttgcccgggcggcctcagtgagcgagcgagcgcgcagagagggagtggccaactccatcactaggggttcctcctaggttaatgattaacccgccatgctacttatctacgtagccatgctctaggatctgaattctagttattaatagtaatcaattacggggtcattagttcatagcccatatatggagttccgcgttacataacttacggtaaatggcccgcctggctgaccgcccaacgacccccgcccattgacgtcaataatgacgtatgttcccatagtaacgccaatagggactttccattgacgtcaatgggtggagtatttacggtaaactgcccacttggcagtacatcaagtgtatcatatgccaagtacgccccctattgacgtcaatgacggtaaatggcccgcctggcattatgcccagtacatgaccttatgggactttcctacttggcagtacatctacgtattagtcatcgctattaccatggtcgaggtgagccccacgttctgcttcactctccccatctcccccccctccccacccccaattttgtatttatttattttttaattattttgtgcagcgatgggggcggggggggggggggggcgcgcgccaggcggggcggggcggggcgaggggcggggcggggcgaggcggagaggtgcggcggcagccaatcagagcggcgcgctccgaaagtttccttttatggcgaggcggcggcggcggcggccctataaaaagcgaagcgcgcggcgggcgggagtcgctgcgaaatgctagcgtttaaacttaagcttaccggtgagctcggatccactagtccagtgtggtggcatgctgcagatatccagcacagtggcggccgcatggtgagcaagggcgaggagctgttcaccggggtggtgcccatcctggtcgagctggacggcgacgtaaacggccacaagttcagcgtgtccggcgagggcgagggcgatgccacctacggcaagctgaccctgaagttcatctgcaccaccggcaagctgcccgtgccctggcccaccctcgtgaccaccctgacctacggcgtgcagtgcttcagccgctaccccgaccacatgaagcagcacgacttcttcaagtccgccatgcccgaaggctacgtccaggagcgcaccatcttcttcaaggacgacggcaactacaagacccgcgccgaggtgaagttcgagggcgacaccctggtgaaccgcatcgagctgaagggcatcgacttcaaggaggacggcaacatcctggggcacaagctggagtacaactacaacagccacaacgtctatatcatggccgacaagcagaagaacggcatcaaggtgaacttcaagatccgccacaacatcgaggacggcagcgtgcagctcgccgaccactaccagcagaacacccccatcggcgacggccccgtgctgctgcccgacaaccactacctgagcacccagtccgccctgagcaaagaccccaacgagaagcgcgatcacatggtcctgctggagttcgtgaccgccgccgggatcactctcggcatggacgagctgtacaagtaactcgagtctagagggcccgtttaaac

SEQ ID NO: 15 - DNA, 4604 bp, synthetic construct
  source 1..4604: mol_type = other DNA
gtcgactagagctcgctgatcagcctcgactgtgccttctagttgccagccatctgttgtttgcccctcccccgtgccttccttgaccctggaaggtgccactcccactgtcctttcctaataaaatgaggaaattgcatcgcattgtctgagtaggtgtcattctattctggggggtggggtggggcaggacagcaagggggaggattggcaagacaatagcaggaaccccactcccacgcgtaggaacccctagtgatggagttggccactccctctctgcgcgctcgctcgctcactgaggccgcccgggcaaagcccgggcgtcgggcgacctttggtcgcccggcctcagtgagcgagcgagcgcgcagagagggagtggccaaggtacctctggccgtcgttttacaacgtcgtgacctctagcttggattctcaccaataaaaaacgcccggcggcaaccgagcgttctgaacaaatccagatggagttctgaggtcattactggatctatcaacaggagtccaagctcagtctactgggcggtttttgcttgcagcacatcccgtcagaccccgtagaaaagatcaaaggatcttcttgagatcctttttttctgcgcgtaatctgctgcttgcaaacaaaaaaaccaccgctaccagcggtggtttgtttgccggatcaagagctaccaactctttttccgaaggtaactggcttcagcagagcgcagataccaaatactgttcttctagtgtagccgtagttaggccaccacttcaagaactctgtagcaccgcctacatacctcgctctgctaatcctgttaccagtggctgctgccagtggcgataagtcgtgtcttaccgggttggactcaagacgatagttaccggataaggcgcagcggtcgggctgaacggggggttcgtgcacacagcccagcttggagcgaacgacctacaccgaactgagatacctacagcgtgagctatgagaaagcgccacgcttcccgaagggagaaaggcggacaggtatccggtaagcggcagggtcggaacaggagagcgcacgagggagcttccagggggaaacgcctggtatctttatagtcctgtcgggtttcgccacctctgacttgagcgtcgatttttgtgatgctcgtcaggggggcggagcctatggaaaaacgccagcaacgcggcctttttacggttcctggccttttgctggccttttgctcacatgttctttcctttcgccagctggcgtaatagcgaagaggcccgcaccgatcgcccttcccaacagttgcgcagcatgaatggcgaatggcgcctgatgcggtattttctccttacgcatctgtgcggtatttcacaccgcatatggtgcactctcagtacaatctgctctgatgccgcatagttaagccagccccgacacccgccaacacccgctgacgcgccctgacgggcttgtctgctcccggcatccgcttacagacaagctgtgaccgacgccgggagctgcatgtgtcagaggttttcaccgtcatcaccgaaacgcgcgatgcagctctggcccgtgtctcaaaatctctgatgttacattgcacaagataaaaatatatcatcatgaacaataaaactgtctgcttacataaacagtaatacaaggggtgttatgagccatattcaacgggaaacgtcgaggccgcgattaaattccaacatggatgctgatttatatgggtataaatgggctcgcgataatgtcgggcaatcaggtgcgacaatctatcgcttgtatgggaagcccgatgcgccagagttgtttctgaaacatggcaaaggtagcgttgccaatgatgttacagatgagatggtcagactaaactggctgacggaatttatgcctcttccgaccatcaagcattttatccgtactcctgatgatgcatggttactcaccactgcgatccccggaaaaacagcattccaggtattagaagaatatcctgattcaggtgaaaatattgttgatgcgctggcagtgttcctgcgccggttgcattcgattcctgtttgtaattgtccttttaacagcgatcgcgtatttcgcctcgctcaggcgcaatcacgaatgaataacggtttggttgatgcgagtgattttgatgacgagcgtaatggctggcctgttgaacaagtctggaaagaaatgcataaacttttgccattctcaccggattcagtcgtcactcatggtgatttctcacttgataaccttatttttgacgaggggaaattaataggttgtattgatgttggacgagtcggaatcgcagaccgataccaggatcttgccatcctatggaactgcctcggtgagttttctccttcattacagaaacggctttttcaaaaatatggtattgataatcctgatatgaataaattgcagtttcatttgatgctcgatgagtttttctaatcagaattggttaattggttgtaacattattcagattgggcttgatttaaaacttcatttttaatttagataaccgtattaccgcctttgagtgagctgataccgctcgccgcagccgaacgaccgttctttcaaataaaacgaaaggctcagtcgaaagactgggcctttcgttttatctgttgtttgtcggtgaacgctctcctgagtaggacaaatccgccgggagcggatttgaacgttgcgaagcaacggcccggagggtggcgggcaggacgcccgccataaactgccaggcatcaaattaagcagaaggccatcctgacggatggcctttttgcgtttctacaaactctgactcttcaggaaacagctatgaccatgattacacccaattgttggccactccctctctgcgcgctcgctcgctcactgaggccgggcgaccaaaggtcgcccgacgcccgggctttgcccgggcggcctcagtgagcgagcgagcgcgcagagagggagtggccaactccatcactaggggttcctcctaggttaatgattaacccgccatgctacttatctacgtagccatgctctaggatctgaattctagttattaatagtaatcaattacggggtcattagttcatagcccatatatggagttccgcgttacataacttacggtaaatggcccgcctggctgaccgcccaacgacccccgcccattgacgtcaataatgacgtatgttcccatagtaacgccaatagggactttccattgacgtcaatgggtggagtatttacggtaaactgcccacttggcagtacatcaagtgtatcatatgccaagtacgccccctattgacgtcaatgacggtaaatggcccgcctggcattatgcccagtacatgaccttatgggactttcctacttggcagtacatctacgtattagtcatcgctattaccatggtcgaggtgagccccacgttctgcttcactctccccatctcccccccctccccacccccaattttgtatttatttattttttaattattttgtgcagcgatgggggcggggggggggggggggcgcgcgccaggcggggcggggcggggcgaggggcggggcggggcgaggcggagaggtgcggcggcagccaatcagagcggcgcgctccgaaagtttccttttatggcgaggcggcggcggcggcggccctataaaaagcgaagcgcgcggcgggcgggagtcgctgcgaaatgctagcgtttaaacttaagcttaccggtgagctcggatccactagtccagtgtggtggcatgctgcagatatccagcacagtggcggccgcatggtgagcaagggcgaggagctgttcaccggggtggtgcccatcctggtcgagctggacggcgacgtaaacggccacaagttcagcgtgtccggcgagggcgagggcgatgccacctacggcaagctgaccctgaagttcatctgcaccaccggcaagctgcccgtgccctggcccaccctcgtgaccaccctgacctacggcgtgcagtgcttcagccgctaccccgaccacatgaagcagcacgacttcttcaagtccgccatgcccgaaggctacgtccaggagcgcaccatcttcttcaaggacgacggcaactacaagacccgcgccgaggtgaagttcgagggcgacaccctggtgaaccgcatcgagctgaagggcatcgacttcaaggaggacggcaacatcctggggcacaagctggagtacaactacaacagccacaacgtctatatcatggccgacaagcagaagaacggcatcaaggtgaacttcaagatccgccacaacatcgaggacggcagcgtgcagctcgccgaccactaccagcagaacacccccatcggcgacggccccgtgctgctgcccgacaaccactacctgagcacccagtccgccctgagcaaagaccccaacgagaagcgcgatcacatggtcctgctggagttcgtgaccgccgccgggatcactctcggcatggacgagctgtacaagtaactcgagtctagagggcccgtttaaac

SEQ ID NO: 16 - DNA, 456 bp, Escherichia coli
  source 1..456: mol_type = other DNA
aaatcccttaacgtgagttttcgttccactgagccctgcgttatcccctgattctgtggataaccgtattaccgcctttgagtgagctgataccgctcgccgcagccgaacgaccgagcgcagcgagtcagtgagcgaggaagcggaagagcgcccaatacgcaaaccgcctctccccgcgcgttggccgattcattaatgcagctggcacgacaggtttcccgactggaaagcgggcagtgatctggcgtaccgttcctgtctaaaatccctttaatcggcctcctgtttagctcccgctctgattctaacgaggaaagcacgttatacgtgctcgtcaaagcgttgatattcagtcaattacaaacattaataacgaagagatgacagaaaaattttcattctgtgacagagaaaaagtagccgaagatgacggtttgtcacatggagttggca

SEQ ID NO: 17 - DNA, 4672 bp, synthetic construct
  source 1..4672: mol_type = other DNA
gtcgactagagctcgctgatcagcctcgactgtgccttctagttgccagccatctgttgtttgcccctcccccgtgccttccttgaccctggaaggtgccactcccactgtcctttcctaataaaatgaggaaattgcatcgcattgtctgagtaggtgtcattctattctggggggtggggtggggcaggacagcaagggggaggattggcaagacaatagcaggaaccccactcccggtaccaggaacccctagtgatggagttggccactccctctctgcgcgctcgctcgctcactgaggccgggcgaccaaaggtcgcccgacgcccgggctttgcccgggcggcctcagtgagcgagcgagcgcgcagctgcctgcaggactagttgatgcggtattttctccttacgcatctgtgcggtatttcacaccgcatacgtcacatgtgtcagaggttttcaccgtcatcaccgaacactgagcgtcagaccccgtagaaaagatcaaaggatcttcttgagatcctttttttctgcgcgtaatctgctgcttgcaaacaaaaaaaccaccgctaccagcggtggtttgtttgccggatcaagagctaccaactctttttccgaaggtaactggcttcagcagagcgcagataccaaatactgtccttctagtgtagccgtagttaggccaccacttcaagaactctgtagcaccgcctacatacctcgctctgctaatcctgttaccagtggctgctgccagtggcgataagtcgtgtcttaccgggttggactcaagacgatagttaccggataaggcgcagcggtcgggctgaacggggggttcgtgcacacagcccagcttggagcgaacgacctacaccgaactgagatacctacagcgtgagctatgagaaagcgccacgcttcccgaagggagaaaggcggacaggtatccggtaagcggcagggtcggaacaggagagcgcacgagggagcttccagggggaaacgcctggtatctttatagtcctgtcgggtttcgccacctctgacttgagcgtcgatttttgtgatgctcgtcaggggggcggagcctatggaaaaacgccagcaacgcggcctttttacggttcctggccttttgctggccttttgctcacatgtacgcgcgagtcgaaagggcctcgtgatacgcctatttttataggttaatgtgatgataataatggtttcttagacgtcaggtggcacttttcggggaaatgtgcgcggaacccctatttgtttatttttctaaatacattcaaatatgtatccgctcatgagacaataaccctgataaatgcttcaataatattgaaaaaggaagagtatgagtattcaacatttccgtgtcgcccttattcccttttttgcggcattttgccttcctgtttttgctcacccagaaacgctggtgaaagtaaaagatgctgaagatcagttgggtgcacgagtgggttacatcgaactggatctcaacagcggtaagatccttgagagttttcgccccgaagaacgttttccaatgatgagcacttttaaagttctgctatgtggcgcggtattatcccgtattgacgccgggcaagagcaactcggtcgccgcatacactattctcagaatgacttggttgagtactcaccagtcacagaaaagcatcttacggatggcatgacagtaagagaattatgcagtgctgccataaccatgagtgataacactgcggccaacttacttctgacaacgatcggaggaccgaaggagctaaccgcttttttgcacaacatgggggatcatgtaactcgccttgatcgttgggaaccggagctgaatgaagccataccaaacgacgagcgtgacaccacgatgcctgtagcaatggcaacaacgttgcgcaaactattaactggcgaactacttactctagcttcccggcaacaattaatagactggatggaggcggataaagttgcaggaccacttctgcgctcggcgcttccggctggctggtttattgctgataaatctggagccggtgagcgtggatctcgcggtatcattgcagcactggggccagatggtaagccctcccgtatcgtagttatctacaccacggggagtcaggcaactatggatgaacgaaatagacagatcgctgagataggtgcctcactgattaagcattggtaactgtcagaccaagtttactcatatatactttagattgatttaaaacttcatttttaatttaaaaggatctaggtgaagatcctttttgataatctcatgaccaaaatcccttaacgtgagttttcgttccactgagcgtcagtttatcccttaaccctgcgttatcccctgattctgtggataaccgtattaccgcctttgagtgagctgataccgctcgccgcagccgaacgaccgagcgcagcgagtcagtgagcgaggaagcggaagaacgcccaatacgcaaaccgcctctccccgcgcgttggccgattcattaatgcagctggcacgacaggtttcccgactggaaagcgggcagtgatctggcgtaccgttcctgtctaaaatccctttaatcggcctcctgtttagctcccgctctgattctaacgaggaaagcacgttatacgtgctcgtcaaagcgttgatattcagtcaattacaaacattaataacgaagagatgacagaaaaattttcattctgtgacagagaaaaagtagccgaagatgtcggtttgtcacatggagttggcatatggtgcactctcagtacaatctgctctgatgccgcatagttaagccagccccgacacccgccaacacccgctgacgcgccctgacgggcttgtctgaagcaaccatagtctcccggcatccgcttacagacaagctgtgaccgtctacgggagctgaacaattgcctgcaggcagctgcgcgctcgctcgctcactgaggccgcccgggcgtcgggcgacctttggtcgcccggcctcagtgagcgagcgagcgcgcagagagggagtggccaactccatcactaggggttcctacgcgtttaatgattaacccgccatgctacttatctacgtagccatgctctaggatctgaattctagttattaatagtaatcaattacggggtcattagttcatagcccatatatggagttccgcgttacataacttacggtaaatggcccgcctggctgaccgcccaacgacccccgcccattgacgtcaataatgacgtatgttcccatagtaacgccaatagggactttccattgacgtcaatgggtggagtatttacggtaaactgcccacttggcagtacatcaagtgtatcatatgccaagtacgccccctattgacgtcaatgacggtaaatggcccgcctggcattatgcccagtacatgaccttatgggactttcctacttggcagtacatctacgtattagtcatcgctattaccatggtcgaggtgagccccacgttctgcttcactctccccatctcccccccctccccacccccaattttgtatttatttattttttaattattttgtgcagcgatgggggcggggggggggggggggcgcgcgccaggcggggcggggcggggcgaggggcggggcggggcgaggcggagaggtgcggcggcagccaatcagagcggcgcgctccgaaagtttccttttatggcgaggcggcggcggcggcggccctataaaaagcgaagcgcgcggcgggcgggagtcgctgcgaaatgctagcgtttaaacttaagcttaccggtgagctcggatccatgcatccagtgtggtggcatgctgcagatatccagcacagtggcggccgcatggtgagcaagggcgaggagctgttcaccggggtggtgcccatcctggtcgagctggacggcgacgtaaacggccacaagttcagcgtgtccggcgagggcgagggcgatgccacctacggcaagctgaccctgaagttcatctgcaccaccggcaagctgcccgtgccctggcccaccctcgtgaccaccctgacctacggcgtgcagtgcttcagccgctaccccgaccacatgaagcagcacgacttcttcaagtccgccatgcccgaaggctacgtccaggagcgcaccatcttcttcaaggacgacggcaactacaagacccgcgccgaggtgaagttcgagggcgacaccctggtgaaccgcatcgagctgaagggcatcgacttcaaggaggacggcaacatcctggggcacaagctggagtacaactacaacagccacaacgtctatatcatggccgacaagcagaagaacggcatcaaggtgaacttcaagatccgccacaacatcgaggacggcagcgtgcagctcgccgaccactaccagcagaacacccccatcggcgacggccccgtgctgctgcccgacaaccactacctgagcacccagtccgccctgagcaaagaccccaacgagaagcgcgatcacatggtcctgctggagttcgtgaccgccgccgggatcactctcggcatggacgagctgtacaagtaactcgagtctagagggcccgtttaaac

SEQ ID NO: 18 - DNA, 4672 bp, synthetic construct
  source 1..4672: mol_type = other DNA
gtcgactagagctcgctgatcagcctcgactgtgccttctagttgccagccatctgttgtttgcccctcccccgtgccttccttgaccctggaaggtgccactcccactgtcctttcctaataaaatgaggaaattgcatcgcattgtctgagtaggtgtcattctattctggggggtggggtggggcaggacagcaagggggaggattggcaagacaatagcaggaaccccactcccggtaccaggaacccctagtgatggagttggccactccctctctgcgcgctcgctcgctcactgaggccgggcgaccaaaggtcgcccgacgcccgggctttgcccgggcggcctcagtgagcgagcgagcgcgcagctgcctgcaggactagttgatgcggtattttctccttacgcatctgtgcggtgttctttcaaataaaacgaaaggctcagtcgaaagactgggcctttcgttttatctgttgtttgtcggtgaacgctctcctgagtaggacaaatccgccgggagcggatttgaacgttgcgaagcaacggcccggagggtggcgggcaggacgcccgccataaactgccaggcatcaaattaagcagaaggccatcctgacggatggcctttttgcgtttctacaaactctgactcttgccagccccgacacccgccaacacccgctgacgcgccctgacgggcttgtctgctcccggcatccgcttacagacaagctgtgaccatctccgggagctgcatgtgtcagaggttttcaccgtcatcaccgaacactgagcgtcagaccccgtagaaaagatcaaaggatcttcttgagatcctttttttctgcgcgtaatctgctgcttgcaaacaaaaaaaccaccgctaccagcggtggtttgtttgccggatcaagagctaccaactctttttccgaaggtaactggcttcagcagagcgcagataccaaatactgtccttctagtgtagccgtagttaggccaccacttcaagaactctgtagcaccgcctacatacctcgctctgctaatcctgttaccagtggctgctgccagtggcgataagtcgtgtcttaccgggttggactcaagacgatagttaccggataaggcgcagcggtcgggctgaacggggggttcgtgcacacagcccagcttggagcgaacgacctacaccgaactgagatacctacagcgtgagctatgagaaagcgccacgcttcccgaagggagaaaggcggacaggtatccggtaagcggcagggtcggaacaggagagcgcacgagggagcttccagggggaaacgcctggtatctttatagtcctgtcgggtttcgccacctctgacttgagcgtcgatttttgtgatgctcgtcaggggggcggagcctatggaaaaacgccagcaacgcggcctttttacggttcctggccttttgctggccttttgctcacatgtacgcgcgagtcgaaagggcctcgtgatacgcctatttttataggttaatgtgatgataataatggtttcttagacgtcaggtggcacttttcggggaaatgtgcgcggaacccctatttgtttatttttctaaatacattcaaatatgtatccgctcatgagacaataaccctgataaatgcttcaataatattgaaaaaggaagagtatgagtattcaacatttccgtgtcgcccttattcccttttttgcggcattttgccttcctgtttttgctcacccagaaacgctggtgaaagtaaaagatgctgaagatcagttgggtgcacgagtgggttacatcgaactggatctcaacagcggtaagatccttgagagttttcgccccgaagaacgttttccaatgatgagcacttttaaagttctgctatgtggcgcggtattatcccgtattgacgccgggcaagagcaactcggtcgccgcatacactattctcagaatgacttggttgagtactcaccagtcacagaaaagcatcttacggatggcatgacagtaagagaattatgcagtgctgccataaccatgagtgataacactgcggccaacttacttctgacaacgatcggaggaccgaaggagctaaccgcttttttgcacaacatgggggatcatgtaactcgccttgatcgttgggaaccggagctgaatgaagccataccaaacgacgagcgtgacaccacgatgcctgtagcaatggcaacaacgttgcgcaaactattaactggcgaactacttactctagcttcccggcaacaattaatagactggatggaggcggataaagttgcaggaccacttctgcgctcggcgcttccggctggctggtttattgctgataaatctggagccggtgagcgtggatctcgcggtatcattgcagcactggggccagatggtaagccctcccgtatcgtagttatctacaccacggggagtcaggcaactatggatgaacgaaatagacagatcgctgagataggtgcctcactgattaagcattggtaactgtcagaccaagtttactcatatatactttagattgatttaatggcacgacaggtttcccgactggaaagcgggcagtgatctggcgtaccgttcctgtctaaaatccctttaatcggcctcctgtttagctcccgctctgattctaacgaggaaagcacgttatacgtgctcgtcaactctagcttggattctcaccaataaaaaacgcccggcggcaaccgagcgttctgaacaaatccagatggagttctgaggtcattactggatctatcaacaggagtccaagctcagtctactgggcggtttttacaatctgctctgatgccgcatagttaaaacttcatttttaatttaaaaggatctaggtgaagatcctttttgataatctcatgaccaaaatcccttaacgtgagtttcaattgcctgcaggcagctgcgcgctcgctcgctcactgaggccgcccgggcgtcgggcgacctttggtcgcccggcctcagtgagcgagcgagcgcgcagagagggagtggccaactccatcactaggggttcctacgcgtttaatgattaacccgccatgctacttatctacgtagccatgctctaggatctgaattctagttattaatagtaatcaattacggggtcattagttcatagcccatatatggagttccgcgttacataacttacggtaaatggcccgcctggctgaccgcccaacgacccccgcccattgacgtcaataatgacgtatgttcccatagtaacgccaatagggactttccattgacgtcaatgggtggagtatttacggtaaactgcccacttggcagtacatcaagtgtatcatatgccaagtacgccccctattgacgtcaatgacggtaaatggcccgcctggcattatgcccagtacatgaccttatgggactttcctacttggcagtacatctacgtattagtcatcgctattaccatggtcgaggtgagccccacgttctgcttcactctccccatctcccccccctccccacccccaattttgtatttatttattttttaattattttgtgcagcgatgggggcggggggggggggggggcgcgcgccaggcggggcggggcggggcgaggggcggggcggggcgaggcggagaggtgcggcggcagccaatcagagcggcgcgctccgaaagtttccttttatggcgaggcggcggcggcggcggccctataaaaagcgaagcgcgcggcgggcgggagtcgctgcgaaatgctagcgtttaaacttaagcttaccggtgagctcggatccatgcatccagtgtggtggcatgctgcagatatccagcacagtggcggccgcatggtgagcaagggcgaggagctgttcaccggggtggtgcccatcctggtcgagctggacggcgacgtaaacggccacaagttcagcgtgtccggcgagggcgagggcgatgccacctacggcaagctgaccctgaagttcatctgcaccaccggcaagctgcccgtgccctggcccaccctcgtgaccaccctgacctacggcgtgcagtgcttcagccgctaccccgaccacatgaagcagcacgacttcttcaagtccgccatgcccgaaggctacgtccaggagcgcaccatcttcttcaaggacgacggcaactacaagacccgcgccgaggtgaagttcgagggcgacaccctggtgaaccgcatcgagctgaagggcatcgacttcaaggaggacggcaacatcctggggcacaagctggagtacaactacaacagccacaacgtctatatcatggccgacaagcagaagaacggcatcaaggtgaacttcaagatccgccacaacatcgaggacggcagcgtgcagctcgccgaccactaccagcagaacacccccatcggcgacggccccgtgctgctgcccgacaaccactacctgagcacccagtccgccctgagcaaagaccccaacgagaagcgcgatcacatggtcctgctggagttcgtgaccgccgccgggatcactctcggcatggacgagctgtacaagtaactcgagtctagagggcccgtttaaac

SEQ ID NO: 19 - DNA, 2478 bp, synthetic construct
  source 1..2478: mol_type = other DNA
gttcgcaggtgcggccgcacgcgtctagttattaatagtaatcaattacggggtcattagttcatagcccatatatggagttccgcgttacataacttacggtaaatggcccgcctggctgaccgcccaacgacccccgcccattgacgtcaataatgacgtatgttcccatagtaacgtcaatagggactttccattgacgtcaatgggtggagtatttacggtaaactgcccacttggcagtacatcaagtgtatcatatgccaagtacgccccctattgacgtcaatgacggtaaatggcccgcctggcattatgcccagtacatgaccttatgggactttcctacttggcagtacatctacgtattagtcatcgctattaccatggtgatgcggttttggcagtacatcaatgggcgtggatagcggtttgactcacggggatttccaagtctccaccccattgacgtcaatgggagtttgttttgcaccaaaatcaacgggactttccaaaatgtcgtaacaactccgccccattgacgcaaatgggcggtaggcgtgtacggtgggaggtctatataagcagagctcgtttagtgaaccgtcagatcgcctggagacgccatccacgctgttttgacctccatagaagacaccgggaccgatccagcctccgcggattcgaatcccggccgggaacggtgcattggaacgcggattccccgtgccaagagtgacgtaagtaccgcctatagagtctataggcccacaaaaaatgctttcttcttttaatatacttttttgtttatcttatttctaatactttccctaatctctttctttcagggcaataatgatacaatgtatcatgcctctttgcaccattctaaagaataacagtgataatttctgggttaaggcaatagcaatatttctgcatataaatatttctgcatataaattgtaactgatgtaagaggtttcatattgctaatagcagctacaatccagctaccattctgcttttattttatggttgggataaggctggattattctgagtccaagctaggcccttttgctaatcatgttcatacctcttatcttcctcccacagctcctgggcaacgtgctggtctgtgtgctggcccatcactttggcaaagaattgggattcgaacatcgattgaattcgccgccaccgccaccatggtgagcaagggcgaggagctgttcaccggggtggtgcccatcctggtcgagctggacggcgacgtaaacggccacaagttcagcgtgtccggcgagggcgagggcgatgccacctacggcaagctgaccctgaagttcatctgcaccaccggcaagctgcccgtgccctggcccaccctcgtgaccaccctgacctacggcgtgcagtgcttcagccgctaccccgaccacatgaagcagcacgacttcttcaagtccgccatgcccgaaggctacgtccaggagcgcaccatcttcttcaaggacgacggcaactacaagacccgcgccgaggtgaagttcgagggcgacaccctggtgaaccgcatcgagctgaagggcatcgacttcaaggaggacggcaacatcctggggcacaagctggagtacaactacaacagccacaacgtctatatcatggccgacaagcagaagaacggcatcaaggtgaacttcaagatccgccacaacatcgaggacggcagcgtgcagctcgccgaccactaccagcagaacacccccatcggcgacggccccgtgctgctgcccgacaaccactacctgagcacccagtccgccctgagcaaagaccccaacgagaagcgcgatcacatggtcctgctggagttcgtgaccgccgccgggatcactctcggcatggacgagctgtacaagtgaaagcttgcctcgagcagcgctgctcgagagatctacgggtggcatccctgtgacccctccccagtgcctctcctggccctggaagttgccactccagtgcccaccagccttgtcctaataaaattaagttgcatcattttgtctgactaggtgtccttctataatattatggggtggaggggggtggtatggagcaaggggcaagttgggaagacaacctgtagggcctgcggggtctattgggaaccaagctggagtgcagtggcacaatcttggctcactgcaatctccgcctcctgggttcaagcgattctcctgcctcagcctcccgagttgttgggattccaggcatgcatgaccaggctcagctaatttttgtttttttggtagagacggggtttcaccatattggccaggctggtctccaactcctaatctcaggtgatctacccaccttggcctcccaaattgctgggattacaggcgtgaaccactgctcccttccctgtccttctgattttgtaggtaaccacgtgcacctgcgttc

SEQ ID NO: 20 - DNA, 2897 bp, synthetic construct
  source 1..2897: mol_type = other DNA
gttcgcaggtgcggccggtcgcgtcgacattgattattgactagttattaatagtaatcaattacggggtcattagttcatagcccatatatggagttccgcgttacataacttacggtaaatggcccgcctggctgaccgcccaacgacccccgcccattgacgtcaataatgacgtatgttcccatagtaacgccaatagggactttccattgacgtcaatgggtggagtatttacggtaaactgcccacttggcagtacatcaagtgtatcatatgccaagtacgccccctattgacgtcaatgacggtaaatggcccgcctggcattatgcccagtacatgaccttatgggactttcctacttggcagtacatctacgtattagtcatcgctattaccatggtcgaggtgagccccacgttctgcttcactctccccatctcccccccctccccacccccaattttgtatttatttattttttaattattttgtgcagcgatgggggcggggggggggggggggcgcgcgccaggcggggcggggcggggcgaggggcggggcggggcgaggcggagaggtgcggcggcagccaatcagagcggcgcgctccgaaagtttccttttatggcgaggcggcggcggcggcggccctataaaaagcgaagcgcgcggcgggcgggagtcgctgcgcgctgccttcgccccgtgccccgctccgccgccgcctcgcgccgcccgccccggctctgactgaccgcgttactcccacaggtgagcgggcgggacggcccttctcctccgggctgtaattagcgcttggtttaatgacggcttgtttcttttctgtggctgcgtgaaagccttgaggggctccgggagggccctttgtgcggggggagcggctcggggggtgcgtgcgtgtgtgtgtgcgtggggagcgccgcgtgcggctccgcgctgcccggcggctgtgagcgctgcgggcgcggcgcggggctttgtgcgctccgcagtgtgcgcgaggggagcgcggccgggggcggtgccccgcggtgcggggggggctgcgaggggaacaaaggctgcgtgcggggtgtgtgcgtgggggggtgagcagggggtgtgggcgcgtcggtcgggctgcaaccccccctgcacccccctccccgagttgctgagcacggcccggcttcgggtgcggggctccgtacggggcgtggcgcggggctcgccgtgccgggcggggggtggcggcaggtgggggtgccgggcggggcggggccgcctcgggccggggagggctcgggggaggggcgcggcggcccccggagcgccggcggctgtcgaggcgcggcgagccgcagccattgccttttatggtaatcgtgcgagagggcgcagggacttcctttgtcccaaatctgtgcggagccgaaatctgggaggcgccgccgcaccccctctagcgggcgcggggcgaagcggtgcggcgccggcaggaaggaaatgggcggggagggccttcgtgcgtcgccgcgccgccgtccccttctccctctccagcctcggggctgtccgcggggggacggctgccttcgggggggacggggcagggcggggttcggcttctggcgtgtgaccggcggctctagagcctctgctaaccatgttcatgccttcttctttttcctacagctcctgggcaacgtgctggttattgtgctgtctcatcattttggcaaaggatccggtaccgaggagatctgccgccgcgatcgccatggtgagcaagggcgaggagctgttcaccggggtggtgcccatcctggtcgagctggacggcgacgtaaacggccacaagttcagcgtgtccggcgagggcgagggcgatgccacctacggcaagctgaccctgaagttcatctgcaccaccggcaagctgcccgtgccctggcccaccctcgtgaccaccctgacctacggcgtgcagtgcttcagccgctaccccgaccacatgaagcagcacgacttcttcaagtccgccatgcccgaaggctacgtccaggagcgcaccatcttcttcaaggacgacggcaactacaagacccgcgccgaggtgaagttcgagggcgacaccctggtgaaccgcatcgagctgaagggcatcgacttcaaggaggacggcaacatcctggggcacaagctggagtacaactacaacagccacaacgtctatatcatggccgacaagcagaagaacggcatcaaggtgaacttcaagatccgccacaacatcgaggacggcagcgtgcagctcgccgaccactaccagcagaacacccccatcggcgacggccccgtgctgctgcccgacaaccactacctgagcacccagtccgccctgagcaaagaccccaacgagaagcgcgatcacatggtcctgctggagttcgtgaccgccgccgggatcactctcggcatggacgagctgtacaagtaaacgcgtacgcggccgctcgaggattataaggatgacgacgataaattcgtcgagcaccaccaccaccaccactaataaggtttatccgatccaccggatctagataagatatccgatccaccggatctagataactgatcataatcagccataccacatttgtagaggttttacttgctttaaaaaacctcccacacctccccctgaacctgaaacataaaatgaatgcaattgttgttgttaacttgtttattgcagcttataatggttacaaataaagcaatagcatcacaaatttcacaaataaagcatttttttcactgcattctagttgtggtttgtccaaactcatcaatgtatcttaacgcggtaaccacgtgcacctgcgttc

SEQ ID NO: 21 - DNA, 3867 bp, synthetic construct
  source 1..3867: mol_type = other DNA
gttcgcaggtgcggccgcacgcgtctagttattaatagtaatcaattacggggtcattagttcatagcccatatatggagttccgcgttacataacttacggtaaatggcccgcctggctgaccgcccaacgacccccgcccattgacgtcaataatgacgtatgttcccatagtaacgccaatagggactttccattgacgtcaatgggtggagtatttacggtaaactgcccacttggcagtacatcaagtgtatcatatgccaagtacgccccctattgacgtcaatgacggtaaatggcccgcctggcattatgcccagtacatgaccttatgggactttcctacttggcagtacatctacgtattagtcatcgctattaccatggtgatgcggttttggcagtacatcaatgggcgtggatagcggtttgactcacggggatttccaagtctccaccccattgacgtcaatgggagtttgttttggcaccaaaatcaacgggactttccaaaatgtcgtaacaactccgccccattgacgcaaatgggcggtaggcgtgtacggtgggaggtctatataagcagagctcgtttagtgaaccgtcagatcgcctggagacgccatccacgctgttttgacctccatagaagacaccgggaccgatccagcctccgcggattcgaatcccggccgggaacggtgcattggaacgcggattccccgtgccaagagtgacgtaagtaccgcctatagagtctataggcccacaaaaaatgctttcttcttttaatatacttttttgtttatcttatttctaatactttccctaatctctttctttcagggcaataatgatacaatgtatcatgcctctttgcaccattctaaagaataacagtgataatttctgggttaaggcaatagcaatatttctgcatataaatatttctgcatataaattgtaactgatgtaagaggtttcatattgctaatagcagctacaatccagctaccattctgcttttattttatggttgggataaggctggattattctgagtccaagctaggcccttttgctaatcatgttcatacctcttatcttcctcccacagctcctgggcaacgtgctggtctgtgtgctggcccatcactttggcaaagaattgggattcgaacatcgattgaattctgaatggtggccggacatgcctctggatctccagcctttggaacagccagccacagcaactgcgagcacgaggaaattcacctggccggctctattcagcctcatggcgctctgctggtggtgtccgaacacgaccacagagtgattcaggcctctgccaatgccgccgagttcctgaatctgggctctgtgctgggagtgcctctggccgaaattgacggcgacctgctgatcaagatcctgcctcacctggatcctaccgccgagggaatgcctgtggccgtgcgttgtagaatcggcaaccctagcaccgagtactgcggcctgatgcacagacctccagaaggcggactgatcatcgagctggaaagagctggccccagcatcgatctgtctggaacactggctcccgctctggaaagaatcagaacagccggaagcctgagagccctgtgcgacgatacagtgctgctgttccagcagtgcaccggctacgatagagtgatggtgtacagattcgacgagcaaggccacggcctggtgttctctgaatgtcacgtgcccggcctggaaagctacttcggcaacagataccccagcagcaccgtgcctcagatggccagacagctgtatgtgcggcagcgcgttagagtgctggtggacgtcacataccagcctgtgccactggaacccagactgagccctctgacaggcagagatctggatatgagcggctgcttcctgcggagcatgagcccttgccatctgcagtttctgaaggacatgggcgtcagagccacactggccgtgtctcttgttgttggcggaaagctgtggggcctcgtcgtgtgtcaccactacctgcctcggttcatcagattcgagctgcgggctatctgcaagcggctggccgagagaatcgccaccagaatcacagccctggaatcctgaggatcctctagagtcgacctgcagaagcttgcctcgagcagcgctgctcgagagatctacgggtggcatccctgtgacccctccccagtgcctctcctggccctggaagttgccactccagtgcccaccagccttgtcctaataaaattaagttgcatcattttgtctgactaggtgtccttctataatattatggggtggaggggggtggtatggagcaaggggcaagttgggaagacaacctgtagggcctgcggggtctattgggaaccaagctggagtgcagtggcacaatcttggctcactgcaatctccgcctcctgggttcaagcgattctcctgcctcagcctcccgagttgttgggattccaggcatgcatgaccaggctcagctaatttttgtttttttggtagagacggggtttcaccatattggccaggctggtctccaactcctaatctcaggtgatctacccaccttggcctcccaaattgctgggattacaggcgtgaaccactgctcccttccctgtccttctgattttgtaggtaaccgtgagtagtggaaggcggttctctggccaacgggctgcttgctgctgttagcagttggagaatggatgcctctgcccggtaaagggcacctggggccgcgcccgcagcattcactaactcgtaactctccttcccttcctccaaacacaaaattccatgacactagacaagaaagctgatgcttggaaaagagaattggccttaaatacctagatggactggagagaccatcctttgtggtccatagcttgaggtctgagtaccctgtccccatccacctgcagacctgctgaggctcccctctggctttctcctgcagaaacctctgccatggccaagcctttgtctcaagaagaatccaccctcattgaaagagcaacggctacaatcaacagcatccccatctctgaagactacagcgtcgccagcgcagctctctctagcgacggccgcatcttcactggtgtcaatgtatatcattttactgggggaccttgtgcagaactcgtggtgctgggcactgctgctgctgcggcagctggcaacctgacttgtatcgtcgcgatcggaaatgagaacaggggcatcttgagcccctgcggacggtgtcgacaggtgcttctcgatctgcatcctgggatcaaagcgatagtgaaggacagtgatggacagccgacggcagttgggattcgtgaattgctgccctctggttatgtgtgggagggctaaagagcagaaggaaggggttcgttgttgacttgtggagatgttgaggagaatccaggaccagcaccgggatccatggtgagcggctggcggctgttcaagaagattagcggcggaggtggttctggcggtggaggttcaatgaaccagtccatcccagttgctcccaccccaccccgcagagtgcggctgaagccctggctggtggcccaggtgaacagctgccagtacccagggcttcaatgggtcaacggggaaaagaaattattctgcatcccctggaggcatgccacaaggcatggtcccagccaggacggagataacaccatcttcaaggtaagccccggggaggaggttggctggacctccagggcaccctgtccccagaagaggagcgcacataacgcacacaggcagctcctcgaggcacctgcgttc

SEQ ID NO: 22 - DNA, 4317 bp, synthetic construct
  source 1..4317: mol_type = other DNA
gttcgcaggtgcagtccatcacgagcagctggtttctaagatgctatttcccgtataaagcatgagaccgtgacttgccagccccacagagccccgcccttgtccatcactggcatctggactccagcctgggttggggcaaagagggaaatgagatcatgtcctaaccctgatcctcttgtcccacagatatccagaaccctgaccctgctgcggccgccaccatggacttccaggtgcagatcttcagcttcctgctgatcagcgccagcgtgatcatgagccggatggccgacatccagatgacccagagcccttcctctctttccgcttccgtgggggacagggtaactattacctgccgagcttcccagggcatccgcaactacctcgcatggtaccagcagaagcctggcaaagctcccaagctgctgatctacgcagcttcgaccctgcagagcggtgtcccctctcgcttcagtggatctggatctggtacggactttactctgaccatctcgtccctgcagccggaagatgtggccacttattactgtcagcgttacaaccgcgcgccctataccttcggccagggcaccaaggttgagatcaagggaggctccagccgttcttcgtcctctggggggggtggctccggcggtggtggttccgaggtgcagctggtggagagcggcggagggctggtgcagccagggcgctcgttgcgcctgtcatgcgccgcttctggcttcacatttgatgactacgccatgcattgggtccgccaggcccccggcaagggcctggagtgggtcagcgccatcacctggaactccggccacattgactacgcggacagcgtggagggcagattcaccatctcccgtgacaacgcgaaaaacagcctttacttgcagatgaattccctgcgggctgaggacaccgccgtgtactactgtgccaaggtgagctacctgtctacggccagttcgttggattattggggccaaggcactctcgtcaccgtgagcagtctcgagcagaagctgatcagcgaggaggacctgaaccggatccgtggggtcaccgtctcttcagcgctgagcaactccatcatgtacttcagccacttcgtgccggtcttcctgccagcgaagcccaccacgacgccagcgccgcgaccaccaacaccggcgcccaccatcgcgtcgcagcccctgtccctgcgcccagaggcgtgccggccagcggcggggggcgcagtgcacacgagggggctggacccctttgggttttgggtgctggtggtggttggtggagtcctggcttgctatagcttgctagtaacagtggcctttattattttctgggtgaggagtaagaggagcaggctcctgcacagtgactacatgaacatgactccccgccgccccgggcccacccgcaagcattaccagccctatgccccaccacgcgacttcgcagcctatcgctccctcgagagagtgagagtgaagttcagcaggagcgcagacgcccccgcgtaccagcagggccagaaccagctctataacgagctcaatctaggacgaagagaggagtacgatgttttggacaagagacgtggccgggaccctgagatggggggaaagccgagaaggaagaaccctcaggaaggcctgtacaatgaactgcagaaagataagatggcggaggcctacagtgagattgggatgaaaggcgagcgccggaggggcaaggggcacgatggcctttaccagggtctcagtacagccaccaaggacacctacgacgcccttcacatgcaggccctgccccctcgcggttccggagccacgaacttctctctgttaaagcaagcaggagacgtggaagaaaaccccggtcccggttccggagagggcagaggaagcttgctcacctgcggggatgtggaggagaatccaggtcctatgcacagctcagcactgctctgttgcctggtcctcctgactggggtgagggccagcccaggccagggcacccagtctgagaacagctgcacccacttcccaggcaacctgcctaacatgcttcgagatctccgagatgccttcagcagagtgaagactttctttcaaatgaaggatcagctggacaacttgttgttaaaggagtccttgctggaggactttaagggttacctgggttgccaagccttgtctgagatgatccagttttacctggaggaggtgatgccccaagctgagaaccaagacccagacatcaaggcgcatgtgaactccctgggggagaacctgaagaccctcaggctgaggctacggcgctgtcatcgatttcttccctgtgaaaacaagagcaaggccgtggagcaggtgaagaatgcctttaataagctccaagagaaaggcatctacaaagccatgagtgagtttgacatcttcatcaactacatagaagcctacatgacaatgaagatacgaaacggttccggagccacgaacttctctctgttaaagcaagcaggagacgtggaagaaaaccccggtcccggttccggagagggcagaggaagcttgctcacctgcggggatgtggaggagaatccaggtcctatgccgccctccgggctgcggctgctgctgctgctgctaccgctgctgtggctactggtgctgacgcctggccggccggccgcgggactatccacctgcaagactatcgacatggagctggtgaagcggaagcgcatcgaggccatccgcggccagatcctgtccaagctgcggctcgccagccccccgagccagggggaggtgccgcccggcccgctgcccgaggccgtgctcgccctgtacaacagcacccgcgaccgggtggccggggagagtgcagaaccggagcccgagcctgaggccgactactacgccaaggaggtcacccgcgtgctaatggtggaaacccacaacgaaatctatgacaagttcaagcagagtacacacagcatatatatgttcttcaacacatcagagctccgagaagcggtacctgaacccgtgttgctctcccgggcagagctgcgtctgctgaggctcaagttaaaagtggagcagcacgtggagctgtaccagaaatacagcaacaattcctggcgatacctcagcaaccggctgctggcacccagcgactcgccagagtggttatcttttgatgtcaccggagttgtgcggcagtggttgagccgtggaggggaaattgagggctttcaccttagcgcccactgctccagagacagcagggataacacactgcaagtggacatcaacgggttcactaccggccgccgaggtgacctggccaccattcatggcatgaaccggcctttcctgcttctcatggccaccccgctggagagggcccagcatctgcaaagctcccggcaccgccgagccctggacaccaactattgcttcagctccacggagaagaactgctgcgtgcggcagctgtacattgacttccgcaaggacctcggctggaagtggatccacgagcccaagggctaccatgccaacttctgcctcgggccctgcccctacatttggagcctggacacgcagtacagcaaggtcctggccctgtacaaccagcataacccgggcgcctcggcggcgccgtgctgcgtgccgcaggcgctggagccgctgcccatcgtgtactacgtgggccgcaagcccaaggtggagcagctgtccaacatgatcgtgcgctcctgcaagtgcagctgacctcgactgtgccttctagttgccagccatctgttgtttgcccctcccccgtgccttccttgaccctggaaggtgccactcccactgtcctttcctaataaaatgaggaaattgcatcgcattgtctgagtaggtgtcattctattctggggggtggggtggggcaggacagcaagggggaggattgggaagacaatagcaggcatgctggggatgcggtgggctctatggcttctgaggcggaaagaaccagctggggctctagggggtatccccactagtcgtgtaccagctgagagactctaaatccagtgacaagtctgtctgcctattcaccgattttgattctcaaacaaatgtgtcacaaagtaaggattctgatgtgtatatcacagacaaaactgtgctagacatgaggtctatggacttcaagagcaacagtgctgtggcctggagcaacaaatctgactttgcatgtgcaaacgccttcaaagatccacctgcgttc

SEQ ID NO: 23 - DNA, 589 bp, Escherichia coli
  source 1..589: mol_type = other DNA
ttgagatcctttttttctgcgcgtaatctgctgcttgcaaacaaaaaaaccaccgctaccagcggtggtttgtttgccggatcaagagctaccaactctttttccgaaggtaactggcttcagcagagcgcagataccaaatactgttcttctagtgtagccgtagttaggccaccacttcaagaactctgtagcaccgcctacatacctcgctctgctaatcctgttaccagtggctgctgccagtggcgataagtcgtgtcttaccgggttggactcaagacgatagttaccggataaggcgcagcggtcgggctgaacggggggttcgtgcacacagcccagcttggagcgaacgacctacaccgaactgagatacctacagcgtgagctatgagaaagcgccacgcttcccgaagggagaaaggcggacaggtatccggtaagcggcagggtcggaacaggagagcgcacgagggagcttccagggggaaacgcctggtatctttatagtcctgtcgggtttcgccacctctgacttgagcgtcgatttttgtgatgctcgtcaggggggcggagcctatggaaa

SEQ ID NO: 24 - DNA, 87 bp, Escherichia coli
  source 1..87: mol_type = genomic DNA
caaataaaacgaaaggctcagtcgaaagactgggcctttcgttttatctgttgtttgtcggtgaacgctctcctgagtaggacaaat

SEQ ID NO: 25 - DNA, 88 bp, Escherichia coli
  source 1..88: mol_type = genomic DNA
tggcgggcaggacgcccgccataaactgccaggcatcaaattaagcagaaggccatcctgacggatggcctttttgcgtttctacaaa

SEQ ID NO: 26 - DNA, 95 bp, Escherichia coli
  source 1..95: mol_type = genomic DNA
attctcaccaataaaaaacgcccggcggcaaccgagcgttctgaacaaatccagatggagttctgaggtcattactggatctatcaacaggagtc

SEQ ID NO: 27 - DNA, 961 bp, synthetic construct
  source 1..961: mol_type = other DNA
gctagcgtttctgcacacttaagcttgagacgggtaccgagctcggatccgaattctgcagatatccagcacagtggcggccgctcgagtgtgcagtgtgagcaagggcgaggagctgttcaccggggtggtgcccatcctggtcgagctggacggcgacgtaaacggccacaagttcagcgtgtccggcgagggcgagggcgatgccacctacggcaagctgaccctgaagttcatctgcaccaccggcaagctgcccgtgccctggcccaccctcgtgaccaccctgacctacggcgtgcagtgcttcagccgctaccccgaccacatgaagcagcacgacttcttcaagtccgccatgcccgaaggctacgtccaggagcgcaccatcttcttcaaggacgacggcaactacaagacccgcgccgaggtgaagttcgagggcgacaccctggtgaaccgcatcgagctgaagggcatcgacttcaaggaggacggcaacatcctggggcacaagctggagtacaactacaacagccacaacgtctatatcatggccgacaagcagaagaacggcatcaaggtgaacttcaagatccgccacaacatcgaggacggcagcgtgcagctcgccgaccactaccagcagaacacccccatcggcgacggccccgtgctgctgcccgacaaccactacctgagcacccagtccgccctgagcaaagaccccaacgagaagcgcgatcacatggtcctgctggagttcgtgaccgccgccgggatcactctcggcatggacgagctgtacaagacgtctcactagtaaaaaaaaaaaaaaaaaaaaaaaaaaaaaaaaaaaaaaaaaaaaaaaaaaaaaaaaaaaaaaaaaaaaaaaaaaaaaaaaaaaaaaaaaaaaaaaaaaaaggaagagcctagctacctactcgagtctagagggccc

SEQ ID NO: 28 - DNA, 247 bp, synthetic construct
  source 1..247: mol_type = other DNA
gctagcgtttctgcacacttaagcttgagacgggtaccgagctcggatccgaattctgcagatatccagcacagtggcggccgctcgagtgtgcagtacgtctcactagtaaaaaaaaaaaaaaaaaaaaaaaaaaaaaaaaaaaaaaaaaaaaaaaaaaaaaaaaaaaaaaaaaaaaaaaaaaaaaaaaaaaaaaaaaaaaaaaaaaaaggaagagcctagctacctactcgagtctagagggccc

SEQ ID NO: 29 - DNA, 1012 bp, synthetic construct
  source 1..1012: mol_type = other DNA
taatacgactcactataaggggtcttctggtccccacagactcagagagaacccgccaccatggtgagcaagggcgaggagctgttcaccggggtggtgcccatcctggtcgagctggacggcgacgtaaacggccacaagttcagcgtgtccggcgagggcgagggcgatgccacctacggcaagctgaccctgaagttcatctgcaccaccggcaagctgcccgtgccctggcccaccctcgtgaccaccctgacctacggcgtgcagtgcttcagccgctaccccgaccacatgaagcagcacgacttcttcaagtccgccatgcccgaaggctacgtccaggagcgcaccatcttcttcaaggacgacggcaactacaagacccgcgccgaggtgaagttcgagggcgacaccctggtgaaccgcatcgagctgaagggcatcgacttcaaggaggacggcaacatcctggggcacaagctggagtacaactacaacagccacaacgtctatatcatggccgacaagcagaagaacggcatcaaggtgaacttcaagatccgccacaacatcgaggacggcagcgtgcagctcgccgaccactaccagcagaacacccccatcggcgacggccccgtgctgctgcccgacaaccactacctgagcacccagtccgccctgagcaaagaccccaacgagaagcgcgatcacatggtcctgctggagttcgtgaccgccgccgggatcactctcggcatggacgagctgtacaagtaatagtaagctggagcctcggtggccatgcttcttgccccttgggcctccccccagcccctcctccccttcctgcacccgtacccccgtggtctttgaataaagtctgagtgggcggcaactagtaaaaaaaaaaaaaaaaaaaaaaaaaaaaaaaaaaaaaaaaaaaaaaaaaaaaaaaaaaaaaaaaaaaaaaaaaaaaaaaaaaaaaaaaaaaaaaaaaaaagggaagagc